European Patent Specification EP 3 645 553 B1, published March 15, 2023. Title: Tropism-Modified Recombinant Viral Particles And Uses Thereof For The Targeted Introduction Of Genetic Material Into Human Cells. Applicant: Regeneron Pharmaceuticals, Inc. Sabin, Leah Schoenherr, Christopher Economides, Aris N Kyratsous, Christos Murphy, Andrew  J. The sequence listing filed with the application follows.

SEQUENCE LISTING (55 sequences)

SEQ ID NO: 1 - protein, 13 aa, Artificial Sequence
  SpyTag
AHIVMVDAYKPTK

SEQ ID NO: 2 - protein, 10 aa, Artificial Sequence
  KTag
ATHIKFSKRD

SEQ ID NO: 3 - protein, 113 aa, Artificial Sequence
  Spycatcher
VDTLSGLSSEQGQSGDMTIEEDSATHIKFSKRDEDGKELAGATMELRDSSGKTISTWISDGQVKDFYLYPGKYTFVETAAPDGYEVATAITFTVNEQGQVTVNGKATKGDAHI

SEQ ID NO: 4 - protein, 108 aa, Artificial Sequence
  SpyLigase
MSYYHHHHHHDYDGQSGDGKELAGATMELRDSSGKTISTWISDGQVKDFYLYPGKYTFVETAAPDGYEVATAITFTVNEQGQVTVNGKATKGGSGGSGGSGEDSATHI

SEQ ID NO: 5 - protein, 12 aa, Artificial Sequence
  SnoopTag
KLGDIEFIKVNK

SEQ ID NO: 6 - protein, 133 aa, Artificial Sequence
  SnoopCatcher
MGSSHHHHHHSSGLVPRGSHMKPLRGAVFSLQKQHPDYPDIYGAIDQNGTYQNVRTGEDGKLTFKNLSDGKYRLFENSEPAGYKPVQNKPIVAFQIVNGEVRDVTSIVPQDIPATYEFTNGKHYITNEPIPPK

SEQ ID NO: 7 - protein, 16 aa, Artificial Sequence
  Isopeptag
TDKDMTITFTNKKDAE

SEQ ID NO: 8 - DNA, 2208 bp, Artificial Sequence
  pAAV2-CAP wt DNA
atggctgccgatggttatcttccagattggctcgaggacactctctctgaaggaataagacagtggtggaagctcaaacctggcccaccaccaccaaagcccgcagagcggcataaggacgacagcaggggtcttgtgcttcctgggtacaagtacctcggacccttcaacggactcgacaagggagagccggtcaacgaggcagacgccgcggccctcgagcacgacaaagcctacgaccggcagctcgacagcggagacaacccgtacctcaagtacaaccacgccgacgcggagtttcaggagcgccttaaagaagatacgtcttttgggggcaacctcggacgagcagtcttccaggcgaaaaagagggttcttgaacctctgggcctggttgaggaacctgttaagacggctccgggaaaaaagaggccggtagagcactctcctgtggagccagactcctcctcgggaaccggaaaggcgggccagcagcctgcaagaaaaagattgaattttggtcagactggagacgcagactcagtacctgacccccagcctctcggacagccaccagcagccccctctggtctgggaactaatacgatggctacaggcagtggcgcaccaatggcagacaataacgagggcgccgacggagtgggtaattcctcgggaaattggcattgcgattccacatggatgggcgacagagtcatcaccaccagcacccgaacctgggccctgcccacctacaacaaccacctctacaaacaaatttccagccaatcaggagcctcgaacgacaatcactactttggctacagcaccccttgggggtattttgacttcaacagattccactgccacttttcaccacgtgactggcaaagactcatcaacaacaactggggattccgacccaagagactcaacttcaagctctttaacattcaagtcaaagaggtcacgcagaatgacggtacgacgacgattgccaataaccttaccagcacggttcaggtgtttactgactcggagtaccagctcccgtacgtcctcggctcggcgcatcaaggatgcctcccgccgttcccagcagacgtcttcatggtgccacagtatggatacctcaccctgaacaacgggagtcaggcagtaggacgctcttcattttactgcctggagtactttccttctcagatgctgcgtaccggaaacaactttaccttcagctacacttttgaggacgttcctttccacagcagctacgctcacagccagagtctggaccgtctcatgaatcctctcatcgaccagtacctgtattacttgagcagaacaaacactccaagtggaaccaccacgcagtcaaggcttcagttttctcaggccggagcgagtgacattcgggaccagtctaggaactggcttcctggaccctgttaccgccagcagcgagtatcaaagacatctgcggataacaacaacagtgaatactcgtggactggagctaccaagtaccacctcaatggcagagactctctggtgaatccgggcccggccatggcaagccacaaggacgatgaagaaaagttttttcctcagagcggggttctcatctttgggaagcaaggctcagagaaaacaaatgtggacattgaaaaggtcatgattacagacgaagaggaaatcaggacaaccaatcccgtggctacggagcagtatggttctgtatctaccaacctccagagaggcaacagacaagcagctaccgcagatgtcaacacacaaggcgttcttccaggcatggtctggcaggacagagatgtgtaccttcaggggcccatctgggcaaagattccacacacggacggacattttcacccctctcccctcatgggtggattcggacttaaacaccctcctccacagattctcatcaagaacaccccggtacctgcgaatccttcgaccaccttcagtgcggcaaagtttgcttccttcatcacacagtactccacgggacaggtcagcgtggagatcgagtgggagctgcagaaggaaaacagcaaacgctggaatcccgaaattcagtacacttccaactacaacaagtctgttaatgtggactttactgtggacactaatggcgtgtattcagagcctcgccccattggcaccagatacctgactcgtaatctgtaa

SEQ ID NO: 9 - protein, 735 aa, adeno-associated virus 2 [sequence omitted]

SEQ ID NO: 10 - DNA, 2208 bp, Artificial Sequence
  pAAV2-CAP R585A R588A (HBM) DNA
atggctgccgatggttatcttccagattggctcgaggacactctctctgaaggaataagacagtggtggaagctcaaacctggcccaccaccaccaaagcccgcagagcggcataaggacgacagcaggggtcttgtgcttcctgggtacaagtacctcggacccttcaacggactcgacaagggagagccggtcaacgaggcagacgccgcggccctcgagcacgacaaagcctacgaccggcagctcgacagcggagacaacccgtacctcaagtacaaccacgccgacgcggagtttcaggagcgccttaaagaagatacgtcttttgggggcaacctcggacgagcagtcttccaggcgaaaaagagggttcttgaacctctgggcctggttgaggaacctgttaagacggctccgggaaaaaagaggccggtagagcactctcctgtggagccagactcctcctcgggaaccggaaaggcgggccagcagcctgcaagaaaaagattgaattttggtcagactggagacgcagactcagtacctgacccccagcctctcggacagccaccagcagccccctctggtctgggaactaatacgatggctacaggcagtggcgcaccaatggcagacaataacgagggcgccgacggagtgggtaattcctcgggaaattggcattgcgattccacatggatgggcgacagagtcatcaccaccagcacccgaacctgggccctgcccacctacaacaaccacctctacaaacaaatttccagccaatcaggagcctcgaacgacaatcactactttggctacagcaccccttgggggtattttgacttcaacagattccactgccacttttcaccacgtgactggcaaagactcatcaacaacaactggggattccgacccaagagactcaacttcaagctctttaacattcaagtcaaagaggtcacgcagaatgacggtacgacgacgattgccaataaccttaccagcacggttcaggtgtttactgactcggagtaccagctcccgtacgtcctcggctcggcgcatcaaggatgcctcccgccgttcccagcagacgtcttcatggtgccacagtatggatacctcaccctgaacaacgggagtcaggcagtaggacgctcttcattttactgcctggagtactttccttctcagatgctgcgtaccggaaacaactttaccttcagctacacttttgaggacgttcctttccacagcagctacgctcacagccagagtctggaccgtctcatgaatcctctcatcgaccagtacctgtattacttgagcagaacaaacactccaagtggaaccaccacgcagtcaaggcttcagttttctcaggccggagcgagtgacattcgggaccagtctaggaactggcttcctggaccctgttaccgccagcagcgagtatcaaagacatctgcggataacaacaacagtgaatactcgtggactggagctaccaagtaccacctcaatggcagagactctctggtgaatccgggcccggccatggcaagccacaaggacgatgaagaaaagttttttcctcagagcggggttctcatctttgggaagcaaggctcagagaaaacaaatgtggacattgaaaaggtcatgattacagacgaagaggaaatcaggacaaccaatcccgtggctacggagcagtatggttctgtatctaccaacctccaggcgggcaacgcgcaagcagctaccgcagatgtcaacacacaaggcgttcttccaggcatggtctggcaggacagagatgtgtaccttcaggggcccatctgggcaaagattccacacacggacggacattttcacccctctcccctcatgggtggattcggacttaaacaccctcctccacagattctcatcaagaacaccccggtacctgcgaatccttcgaccaccttcagtgcggcaaagtttgcttccttcatcacacagtactccacgggacaggtcagcgtggagatcgagtgggagctgcagaaggaaaacagcaaacgctggaatcccgaaattcagtacacttccaactacaacaagtctgttaatgtggactttactgtggacactaatggcgtgtattcagagcctcgccccattggcaccagatacctgactcgtaatctgtaa

SEQ ID NO: 11 - protein, 735 aa, Artificial Sequence
  pAAV2-CAP R585A R588A (HBM) AA
MAADGYLPDWLEDTLSEGIRQWWKLKPGPPPPKPAERHKDDSRGLVLPGYKYLGPFNGLDKGEPVNEADAAALEHDKAYDRQLDSGDNPYLKYNHADAEFQERLKEDTSFGGNLGRAVFQAKKRVLEPLGLVEEPVKTAPGKKRPVEHSPVEPDSSSGTGKAGQQPARKRLNFGQTGDADSVPDPQPLGQPPAAPSGLGTNTMATGSGAPMADNNEGADGVGNSSGNWHCDSTWMGDRVITTSTRTWALPTYNNHLYKQISSQSGASNDNHYFGYSTPWGYFDFNRFHCHFSPRDWQRLINNNWGFRPKRLNFKLFNIQVKEVTQNDGTTTIANNLTSTVQVFTDSEYQLPYVLGSAHQGCLPPFPADVFMVPQYGYLTLNNGSQAVGRSSFYCLEYFPSQMLRTGNNFTFSYTFEDVPFHSSYAHSQSLDRLMNPLIDQYLYYLSRTNTPSGTTTQSRLQFSQAGASDIRDQSRNWLPGPCYRQQRVSKTSADNNNSEYSWTGATKYHLNGRDSLVNPGPAMASHKDDEEKFFPQSGVLIFGKQGSEKTNVDIEKVMITDEEEIRTTNPVATEQYGSVSTNLQAGNAQAATADVNTQGVLPGMVWQDRDVYLQGPIWAKIPHTDGHFHPSPLMGGFGLKHPPPQILIKNTPVPANPSTTFSAAKFASFITQYSTGQVSVEIEWELQKENSKRWNPEIQYTSNYNKSVNVDFTVDTNGVYSEPRPIGTRYLTRNL

SEQ ID NO: 12 - DNA, 2244 bp, Artificial Sequence
  pAAV2-CAP N587 SpyTag HBM DNA
atggctgccgatggttatcttccagattggctcgaggacactctctctgaaggaataagacagtggtggaagctcaaacctggcccaccaccaccaaagcccgcagagcggcataaggacgacagcaggggtcttgtgcttcctgggtacaagtacctcggacccttcaacggactcgacaagggagagccggtcaacgaggcagacgccgcggccctcgagcacgacaaagcctacgaccggcagctcgacagcggagacaacccgtacctcaagtacaaccacgccgacgcggagtttcaggagcgccttaaagaagatacgtcttttgggggcaacctcggacgagcagtcttccaggcgaaaaagagggttcttgaacctctgggcctggttgaggaacctgttaagacggctccgggaaaaaagaggccggtagagcactctcctgtggagccagactcctcctcgggaaccggaaaggcgggccagcagcctgcaagaaaaagattgaattttggtcagactggagacgcagactcagtacctgacccccagcctctcggacagccaccagcagccccctctggtctgggaactaatacgatggctacaggcagtggcgcaccaatggcagacaataacgagggcgccgacggagtgggtaattcctcgggaaattggcattgcgattccacatggatgggcgacagagtcatcaccaccagcacccgaacctgggccctgcccacctacaacaaccacctctacaaacaaatttccagccaatcaggagcctcgaacgacaatcactactttggctacagcaccccttgggggtattttgacttcaacagattccactgccacttttcaccacgtgactggcaaagactcatcaacaacaactggggattccgacccaagagactcaacttcaagctctttaacattcaagtcaaagaggtcacgcagaatgacggtacgacgacgattgccaataaccttaccagcacggttcaggtgtttactgactcggagtaccagctcccgtacgtcctcggctcggcgcatcaaggatgcctcccgccgttcccagcagacgtcttcatggtgccacagtatggatacctcaccctgaacaacgggagtcaggcagtaggacgctcttcattttactgcctggagtactttccttctcagatgctgcgtaccggaaacaactttaccttcagctacacttttgaggacgttcctttccacagcagctacgctcacagccagagtctggaccgtctcatgaatcctctcatcgaccagtacctgtattacttgagcagaacaaacactccaagtggaaccaccacgcagtcaaggcttcagttttctcaggccggagcgagtgacattcgggaccagtctaggaactggcttcctggaccctgttaccgccagcagcgagtatcaaagacatctgcggataacaacaacagtgaatactcgtggactggagctaccaagtaccacctcaatggcagagactctctggtgaatccgggcccggccatggcaagccacaaggacgatgaagaaaagttttttcctcagagcggggttctcatctttgggaagcaaggctcagagaaaacaaatgtggacattgaaaaggtcatgattacagacgaagaggaaatcaggacaaccaatcccgtggctacggagcagtatggttctgtatctaccaacctccaggcgggcaacgcccacatcgtgatggtggacgcctacaagccgacgaagcaagcagctaccgcagatgtcaacacacaaggcgttcttccaggcatggtctggcaggacagagatgtgtaccttcaggggcccatctgggcaaagattccacacacggacggacattttcacccctctcccctcatgggtggattcggacttaaacaccctcctccacagattctcatcaagaacaccccggtacctgcgaatccttcgaccaccttcagtgcggcaaagtttgcttccttcatcacacagtactccacgggacaggtcagcgtggagatcgagtgggagctgcagaaggaaaacagcaaacgctggaatcccgaaattcagtacacttccaactacaacaagtctgttaatgtggactttactgtggacactaatggcgtgtattcagagcctcgccccattggcaccagatacctgactcgtaatctgtaa

SEQ ID NO: 13 - protein, 747 aa, Artificial Sequence
  pAAV2-CAP N587 SpyTag HBM AA
MAADGYLPDWLEDTLSEGIRQWWKLKPGPPPPKPAERHKDDSRGLVLPGYKYLGPFNGLDKGEPVNEADAAALEHDKAYDRQLDSGDNPYLKYNHADAEFQERLKEDTSFGGNLGRAVFQAKKRVLEPLGLVEEPVKTAPGKKRPVEHSPVEPDSSSGTGKAGQQPARKRLNFGQTGDADSVPDPQPLGQPPAAPSGLGTNTMATGSGAPMADNNEGADGVGNSSGNWHCDSTWMGDRVITTSTRTWALPTYNNHLYKQISSQSGASNDNHYFGYSTPWGYFDFNRFHCHFSPRDWQRLINNNWGFRPKRLNFKLFNIQVKEVTQNDGTTTIANNLTSTVQVFTDSEYQLPYVLGSAHQGCLPPFPADVFMVPQYGYLTLNNGSQAVGRSSFYCLEYFPSQMLRTGNNFTFSYTFEDVPFHSSYAHSQSLDRLMNPLIDQYLYYLSRTNTPSGTTTQSRLQFSQAGASDIRDQSRNWLPGPCYRQQRVSKTSADNNNSEYSWTGATKYHLNGRDSLVNPGPAMASHKDDEEKFFPQSGVLIFGKQGSEKTNVDIEKVMITDEEEIRTTNPVATEQYGSVSTNLQAGNAHIVMVDAYKPTKQAATADVNTQGVLPGMVWQDRDVYLQGPIWAKIPHTDGHFHPSPLMGGFGLKHPPPQILIKNTPVPANPSTTFSAAKFASFITQYSTGQVSVEIEWELQKENSKRWNPEIQYTSNYNKSVNVDFTVDTNGVYSEPRPIGTRYLTRNL

SEQ ID NO: 14 - DNA, 2253 bp, Artificial Sequence
  pAAV2-CAP N587 Linker 1 SpyTag HBM  DNA
atggctgccgatggttatcttccagattggctcgaggacactctctctgaaggaataagacagtggtggaagctcaaacctggcccaccaccaccaaagcccgcagagcggcataaggacgacagcaggggtcttgtgcttcctgggtacaagtacctcggacccttcaacggactcgacaagggagagccggtcaacgaggcagacgccgcggccctcgagcacgacaaagcctacgaccggcagctcgacagcggagacaacccgtacctcaagtacaaccacgccgacgcggagtttcaggagcgccttaaagaagatacgtcttttgggggcaacctcggacgagcagtcttccaggcgaaaaagagggttcttgaacctctgggcctggttgaggaacctgttaagacggctccgggaaaaaagaggccggtagagcactctcctgtggagccagactcctcctcgggaaccggaaaggcgggccagcagcctgcaagaaaaagattgaattttggtcagactggagacgcagactcagtacctgacccccagcctctcggacagccaccagcagccccctctggtctgggaactaatacgatggctacaggcagtggcgcaccaatggcagacaataacgagggcgccgacggagtgggtaattcctcgggaaattggcattgcgattccacatggatgggcgacagagtcatcaccaccagcacccgaacctgggccctgcccacctacaacaaccacctctacaaacaaatttccagccaatcaggagcctcgaacgacaatcactactttggctacagcaccccttgggggtattttgacttcaacagattccactgccacttttcaccacgtgactggcaaagactcatcaacaacaactggggattccgacccaagagactcaacttcaagctctttaacattcaagtcaaagaggtcacgcagaatgacggtacgacgacgattgccaataaccttaccagcacggttcaggtgtttactgactcggagtaccagctcccgtacgtcctcggctcggcgcatcaaggatgcctcccgccgttcccagcagacgtcttcatggtgccacagtatggatacctcaccctgaacaacgggagtcaggcagtaggacgctcttcattttactgcctggagtactttccttctcagatgctgcgtaccggaaacaactttaccttcagctacacttttgaggacgttcctttccacagcagctacgctcacagccagagtctggaccgtctcatgaatcctctcatcgaccagtacctgtattacttgagcagaacaaacactccaagtggaaccaccacgcagtcaaggcttcagttttctcaggccggagcgagtgacattcgggaccagtctaggaactggcttcctggaccctgttaccgccagcagcgagtatcaaagacatctgcggataacaacaacagtgaatactcgtggactggagctaccaagtaccacctcaatggcagagactctctggtgaatccgggcccggccatggcaagccacaaggacgatgaagaaaagttttttcctcagagcggggttctcatctttgggaagcaaggctcagagaaaacaaatgtggacattgaaaaggtcatgattacagacgaagaggaaatcaggacaaccaatcccgtggctacggagcagtatggttctgtatctaccaacctccaggcgggcaacgcgagcgcccacatcgtgatggtggacgcctacaagccgacgaaggcgcaagcagctaccgcagatgtcaacacacaaggcgttcttccaggcatggtctggcaggacagagatgtgtaccttcaggggcccatctgggcaaagattccacacacggacggacattttcacccctctcccctcatgggtggattcggacttaaacaccctcctccacagattctcatcaagaacaccccggtacctgcgaatccttcgaccaccttcagtgcggcaaagtttgcttccttcatcacacagtactccacgggacaggtcagcgtggagatcgagtgggagctgcagaaggaaaacagcaaacgctggaatcccgaaattcagtacacttccaactacaacaagtctgttaatgtggactttactgtggacactaatggcgtgtattcagagcctcgccccattggcaccagatacctgactcgtaatctgtaa

SEQ ID NO: 15 - protein, 750 aa, Artificial Sequence
  pAAV2-CAP N587 Linker 1 SpyTag HBM  AA
MAADGYLPDWLEDTLSEGIRQWWKLKPGPPPPKPAERHKDDSRGLVLPGYKYLGPFNGLDKGEPVNEADAAALEHDKAYDRQLDSGDNPYLKYNHADAEFQERLKEDTSFGGNLGRAVFQAKKRVLEPLGLVEEPVKTAPGKKRPVEHSPVEPDSSSGTGKAGQQPARKRLNFGQTGDADSVPDPQPLGQPPAAPSGLGTNTMATGSGAPMADNNEGADGVGNSSGNWHCDSTWMGDRVITTSTRTWALPTYNNHLYKQISSQSGASNDNHYFGYSTPWGYFDFNRFHCHFSPRDWQRLINNNWGFRPKRLNFKLFNIQVKEVTQNDGTTTIANNLTSTVQVFTDSEYQLPYVLGSAHQGCLPPFPADVFMVPQYGYLTLNNGSQAVGRSSFYCLEYFPSQMLRTGNNFTFSYTFEDVPFHSSYAHSQSLDRLMNPLIDQYLYYLSRTNTPSGTTTQSRLQFSQAGASDIRDQSRNWLPGPCYRQQRVSKTSADNNNSEYSWTGATKYHLNGRDSLVNPGPAMASHKDDEEKFFPQSGVLIFGKQGSEKTNVDIEKVMITDEEEIRTTNPVATEQYGSVSTNLQAGNASAHIVMVDAYKPTKAQAATADVNTQGVLPGMVWQDRDVYLQGPIWAKIPHTDGHFHPSPLMGGFGLKHPPPQILIKNTPVPANPSTTFSAAKFASFITQYSTGQVSVEIEWELQKENSKRWNPEIQYTSNYNKSVNVDFTVDTNGVYSEPRPIGTRYLTRNL

SEQ ID NO: 16 - DNA, 2256 bp, Artificial Sequence
  pAAV2-CAP N587 Linker 2 SpyTag HBM  DNA
atggctgccgatggttatcttccagattggctcgaggacactctctctgaaggaataagacagtggtggaagctcaaacctggcccaccaccaccaaagcccgcagagcggcataaggacgacagcaggggtcttgtgcttcctgggtacaagtacctcggacccttcaacggactcgacaagggagagccggtcaacgaggcagacgccgcggccctcgagcacgacaaagcctacgaccggcagctcgacagcggagacaacccgtacctcaagtacaaccacgccgacgcggagtttcaggagcgccttaaagaagatacgtcttttgggggcaacctcggacgagcagtcttccaggcgaaaaagagggttcttgaacctctgggcctggttgaggaacctgttaagacggctccgggaaaaaagaggccggtagagcactctcctgtggagccagactcctcctcgggaaccggaaaggcgggccagcagcctgcaagaaaaagattgaattttggtcagactggagacgcagactcagtacctgacccccagcctctcggacagccaccagcagccccctctggtctgggaactaatacgatggctacaggcagtggcgcaccaatggcagacaataacgagggcgccgacggagtgggtaattcctcgggaaattggcattgcgattccacatggatgggcgacagagtcatcaccaccagcacccgaacctgggccctgcccacctacaacaaccacctctacaaacaaatttccagccaatcaggagcctcgaacgacaatcactactttggctacagcaccccttgggggtattttgacttcaacagattccactgccacttttcaccacgtgactggcaaagactcatcaacaacaactggggattccgacccaagagactcaacttcaagctctttaacattcaagtcaaagaggtcacgcagaatgacggtacgacgacgattgccaataaccttaccagcacggttcaggtgtttactgactcggagtaccagctcccgtacgtcctcggctcggcgcatcaaggatgcctcccgccgttcccagcagacgtcttcatggtgccacagtatggatacctcaccctgaacaacgggagtcaggcagtaggacgctcttcattttactgcctggagtactttccttctcagatgctgcgtaccggaaacaactttaccttcagctacacttttgaggacgttcctttccacagcagctacgctcacagccagagtctggaccgtctcatgaatcctctcatcgaccagtacctgtattacttgagcagaacaaacactccaagtggaaccaccacgcagtcaaggcttcagttttctcaggccggagcgagtgacattcgggaccagtctaggaactggcttcctggaccctgttaccgccagcagcgagtatcaaagacatctgcggataacaacaacagtgaatactcgtggactggagctaccaagtaccacctcaatggcagagactctctggtgaatccgggcccggccatggcaagccacaaggacgatgaagaaaagttttttcctcagagcggggttctcatctttgggaagcaaggctcagagaaaacaaatgtggacattgaaaaggtcatgattacagacgaagaggaaatcaggacaaccaatcccgtggctacggagcagtatggttctgtatctaccaacctccaggcgggcaacggcagcgcccacatcgtgatggtggacgcctacaagccgacgaagggcagccaagcagctaccgcagatgtcaacacacaaggcgttcttccaggcatggtctggcaggacagagatgtgtaccttcaggggcccatctgggcaaagattccacacacggacggacattttcacccctctcccctcatgggtggattcggacttaaacaccctcctccacagattctcatcaagaacaccccggtacctgcgaatccttcgaccaccttcagtgcggcaaagtttgcttccttcatcacacagtactccacgggacaggtcagcgtggagatcgagtgggagctgcagaaggaaaacagcaaacgctggaatcccgaaattcagtacacttccaactacaacaagtctgttaatgtggactttactgtggacactaatggcgtgtattcagagcctcgccccattggcaccagatacctgactcgtaatctgtaa

SEQ ID NO: 17 - protein, 751 aa, Artificial Sequence
  pAAV2-CAP N587 Linker 2 SpyTag HBM AA
MAADGYLPDWLEDTLSEGIRQWWKLKPGPPPPKPAERHKDDSRGLVLPGYKYLGPFNGLDKGEPVNEADAAALEHDKAYDRQLDSGDNPYLKYNHADAEFQERLKEDTSFGGNLGRAVFQAKKRVLEPLGLVEEPVKTAPGKKRPVEHSPVEPDSSSGTGKAGQQPARKRLNFGQTGDADSVPDPQPLGQPPAAPSGLGTNTMATGSGAPMADNNEGADGVGNSSGNWHCDSTWMGDRVITTSTRTWALPTYNNHLYKQISSQSGASNDNHYFGYSTPWGYFDFNRFHCHFSPRDWQRLINNNWGFRPKRLNFKLFNIQVKEVTQNDGTTTIANNLTSTVQVFTDSEYQLPYVLGSAHQGCLPPFPADVFMVPQYGYLTLNNGSQAVGRSSFYCLEYFPSQMLRTGNNFTFSYTFEDVPFHSSYAHSQSLDRLMNPLIDQYLYYLSRTNTPSGTTTQSRLQFSQAGASDIRDQSRNWLPGPCYRQQRVSKTSADNNNSEYSWTGATKYHLNGRDSLVNPGPAMASHKDDEEKFFPQSGVLIFGKQGSEKTNVDIEKVMITDEEEIRTTNPVATEQYGSVSTNLQAGNGSAHIVMVDAYKPTKGSQAATADVNTQGVLPGMVWQDRDVYLQGPIWAKIPHTDGHFHPSPLMGGFGLKHPPPQILIKNTPVPANPSTTFSAAKFASFITQYSTGQVSVEIEWELQKENSKRWNPEIQYTSNYNKSVNVDFTVDTNGVYSEPRPIGTRYLTRNL

SEQ ID NO: 18 - DNA, 2268 bp, Artificial Sequence
  pAAV2-CAP N587 Linker 4 SpyTag HBM DNA
atggctgccgatggttatcttccagattggctcgaggacactctctctgaaggaataagacagtggtggaagctcaaacctggcccaccaccaccaaagcccgcagagcggcataaggacgacagcaggggtcttgtgcttcctgggtacaagtacctcggacccttcaacggactcgacaagggagagccggtcaacgaggcagacgccgcggccctcgagcacgacaaagcctacgaccggcagctcgacagcggagacaacccgtacctcaagtacaaccacgccgacgcggagtttcaggagcgccttaaagaagatacgtcttttgggggcaacctcggacgagcagtcttccaggcgaaaaagagggttcttgaacctctgggcctggttgaggaacctgttaagacggctccgggaaaaaagaggccggtagagcactctcctgtggagccagactcctcctcgggaaccggaaaggcgggccagcagcctgcaagaaaaagattgaattttggtcagactggagacgcagactcagtacctgacccccagcctctcggacagccaccagcagccccctctggtctgggaactaatacgatggctacaggcagtggcgcaccaatggcagacaataacgagggcgccgacggagtgggtaattcctcgggaaattggcattgcgattccacatggatgggcgacagagtcatcaccaccagcacccgaacctgggccctgcccacctacaacaaccacctctacaaacaaatttccagccaatcaggagcctcgaacgacaatcactactttggctacagcaccccttgggggtattttgacttcaacagattccactgccacttttcaccacgtgactggcaaagactcatcaacaacaactggggattccgacccaagagactcaacttcaagctctttaacattcaagtcaaagaggtcacgcagaatgacggtacgacgacgattgccaataaccttaccagcacggttcaggtgtttactgactcggagtaccagctcccgtacgtcctcggctcggcgcatcaaggatgcctcccgccgttcccagcagacgtcttcatggtgccacagtatggatacctcaccctgaacaacgggagtcaggcagtaggacgctcttcattttactgcctggagtactttccttctcagatgctgcgtaccggaaacaactttaccttcagctacacttttgaggacgttcctttccacagcagctacgctcacagccagagtctggaccgtctcatgaatcctctcatcgaccagtacctgtattacttgagcagaacaaacactccaagtggaaccaccacgcagtcaaggcttcagttttctcaggccggagcgagtgacattcgggaccagtctaggaactggcttcctggaccctgttaccgccagcagcgagtatcaaagacatctgcggataacaacaacagtgaatactcgtggactggagctaccaagtaccacctcaatggcagagactctctggtgaatccgggcccggccatggcaagccacaaggacgatgaagaaaagttttttcctcagagcggggttctcatctttgggaagcaaggctcagagaaaacaaatgtggacattgaaaaggtcatgattacagacgaagaggaaatcaggacaaccaatcccgtggctacggagcagtatggttctgtatctaccaacctccaggcgggcaacggcctgagcggcgcccacatcgtgatggtggacgcctacaagccgacgaagggcctgagcggccaagcagctaccgcagatgtcaacacacaaggcgttcttccaggcatggtctggcaggacagagatgtgtaccttcaggggcccatctgggcaaagattccacacacggacggacattttcacccctctcccctcatgggtggattcggacttaaacaccctcctccacagattctcatcaagaacaccccggtacctgcgaatccttcgaccaccttcagtgcggcaaagtttgcttccttcatcacacagtactccacgggacaggtcagcgtggagatcgagtgggagctgcagaaggaaaacagcaaacgctggaatcccgaaattcagtacacttccaactacaacaagtctgttaatgtggactttactgtggacactaatggcgtgtattcagagcctcgccccattggcaccagatacctgactcgtaatctgtaa

SEQ ID NO: 19 - protein, 755 aa, Artificial Sequence
  pAAV2-CAP N587 Linker 4 SpyTag HBM  AA
MAADGYLPDWLEDTLSEGIRQWWKLKPGPPPPKPAERHKDDSRGLVLPGYKYLGPFNGLDKGEPVNEADAAALEHDKAYDRQLDSGDNPYLKYNHADAEFQERLKEDTSFGGNLGRAVFQAKKRVLEPLGLVEEPVKTAPGKKRPVEHSPVEPDSSSGTGKAGQQPARKRLNFGQTGDADSVPDPQPLGQPPAAPSGLGTNTMATGSGAPMADNNEGADGVGNSSGNWHCDSTWMGDRVITTSTRTWALPTYNNHLYKQISSQSGASNDNHYFGYSTPWGYFDFNRFHCHFSPRDWQRLINNNWGFRPKRLNFKLFNIQVKEVTQNDGTTTIANNLTSTVQVFTDSEYQLPYVLGSAHQGCLPPFPADVFMVPQYGYLTLNNGSQAVGRSSFYCLEYFPSQMLRTGNNFTFSYTFEDVPFHSSYAHSQSLDRLMNPLIDQYLYYLSRTNTPSGTTTQSRLQFSQAGASDIRDQSRNWLPGPCYRQQRVSKTSADNNNSEYSWTGATKYHLNGRDSLVNPGPAMASHKDDEEKFFPQSGVLIFGKQGSEKTNVDIEKVMITDEEEIRTTNPVATEQYGSVSTNLQAGNGLSGAHIVMVDAYKPTKGLSGQAATADVNTQGVLPGMVWQDRDVYLQGPIWAKIPHTDGHFHPSPLMGGFGLKHPPPQILIKNTPVPANPSTTFSAAKFASFITQYSTGQVSVEIEWELQKENSKRWNPEIQYTSNYNKSVNVDFTVDTNGVYSEPRPIGTRYLTRNL

SEQ ID NO: 20 - DNA, 2280 bp, Artificial Sequence
  pAAV2-CAP N587 Linker 6 SpyTag HBM  DNA
atggctgccgatggttatcttccagattggctcgaggacactctctctgaaggaataagacagtggtggaagctcaaacctggcccaccaccaccaaagcccgcagagcggcataaggacgacagcaggggtcttgtgcttcctgggtacaagtacctcggacccttcaacggactcgacaagggagagccggtcaacgaggcagacgccgcggccctcgagcacgacaaagcctacgaccggcagctcgacagcggagacaacccgtacctcaagtacaaccacgccgacgcggagtttcaggagcgccttaaagaagatacgtcttttgggggcaacctcggacgagcagtcttccaggcgaaaaagagggttcttgaacctctgggcctggttgaggaacctgttaagacggctccgggaaaaaagaggccggtagagcactctcctgtggagccagactcctcctcgggaaccggaaaggcgggccagcagcctgcaagaaaaagattgaattttggtcagactggagacgcagactcagtacctgacccccagcctctcggacagccaccagcagccccctctggtctgggaactaatacgatggctacaggcagtggcgcaccaatggcagacaataacgagggcgccgacggagtgggtaattcctcgggaaattggcattgcgattccacatggatgggcgacagagtcatcaccaccagcacccgaacctgggccctgcccacctacaacaaccacctctacaaacaaatttccagccaatcaggagcctcgaacgacaatcactactttggctacagcaccccttgggggtattttgacttcaacagattccactgccacttttcaccacgtgactggcaaagactcatcaacaacaactggggattccgacccaagagactcaacttcaagctctttaacattcaagtcaaagaggtcacgcagaatgacggtacgacgacgattgccaataaccttaccagcacggttcaggtgtttactgactcggagtaccagctcccgtacgtcctcggctcggcgcatcaaggatgcctcccgccgttcccagcagacgtcttcatggtgccacagtatggatacctcaccctgaacaacgggagtcaggcagtaggacgctcttcattttactgcctggagtactttccttctcagatgctgcgtaccggaaacaactttaccttcagctacacttttgaggacgttcctttccacagcagctacgctcacagccagagtctggaccgtctcatgaatcctctcatcgaccagtacctgtattacttgagcagaacaaacactccaagtggaaccaccacgcagtcaaggcttcagttttctcaggccggagcgagtgacattcgggaccagtctaggaactggcttcctggaccctgttaccgccagcagcgagtatcaaagacatctgcggataacaacaacagtgaatactcgtggactggagctaccaagtaccacctcaatggcagagactctctggtgaatccgggcccggccatggcaagccacaaggacgatgaagaaaagttttttcctcagagcggggttctcatctttgggaagcaaggctcagagaaaacaaatgtggacattgaaaaggtcatgattacagacgaagaggaaatcaggacaaccaatcccgtggctacggagcagtatggttctgtatctaccaacctccaggcgggcaacggcctgagcggcagcggcgcccacatcgtgatggtggacgcctacaagccgacgaagggcctgagcggcagcggccaagcagctaccgcagatgtcaacacacaaggcgttcttccaggcatggtctggcaggacagagatgtgtaccttcaggggcccatctgggcaaagattccacacacggacggacattttcacccctctcccctcatgggtggattcggacttaaacaccctcctccacagattctcatcaagaacaccccggtacctgcgaatccttcgaccaccttcagtgcggcaaagtttgcttccttcatcacacagtactccacgggacaggtcagcgtggagatcgagtgggagctgcagaaggaaaacagcaaacgctggaatcccgaaattcagtacacttccaactacaacaagtctgttaatgtggactttactgtggacactaatggcgtgtattcagagcctcgccccattggcaccagatacctgactcgtaatctgtaa

SEQ ID NO: 21 - protein, 759 aa, Artificial Sequence
  pAAV2-CAP N587 Linker 6 SpyTag HBM  AA
MAADGYLPDWLEDTLSEGIRQWWKLKPGPPPPKPAERHKDDSRGLVLPGYKYLGPFNGLDKGEPVNEADAAALEHDKAYDRQLDSGDNPYLKYNHADAEFQERLKEDTSFGGNLGRAVFQAKKRVLEPLGLVEEPVKTAPGKKRPVEHSPVEPDSSSGTGKAGQQPARKRLNFGQTGDADSVPDPQPLGQPPAAPSGLGTNTMATGSGAPMADNNEGADGVGNSSGNWHCDSTWMGDRVITTSTRTWALPTYNNHLYKQISSQSGASNDNHYFGYSTPWGYFDFNRFHCHFSPRDWQRLINNNWGFRPKRLNFKLFNIQVKEVTQNDGTTTIANNLTSTVQVFTDSEYQLPYVLGSAHQGCLPPFPADVFMVPQYGYLTLNNGSQAVGRSSFYCLEYFPSQMLRTGNNFTFSYTFEDVPFHSSYAHSQSLDRLMNPLIDQYLYYLSRTNTPSGTTTQSRLQFSQAGASDIRDQSRNWLPGPCYRQQRVSKTSADNNNSEYSWTGATKYHLNGRDSLVNPGPAMASHKDDEEKFFPQSGVLIFGKQGSEKTNVDIEKVMITDEEEIRTTNPVATEQYGSVSTNLQAGNGLSGSGAHIVMVDAYKPTKGLSGSGQAATADVNTQGVLPGMVWQDRDVYLQGPIWAKIPHTDGHFHPSPLMGGFGLKHPPPQILIKNTPVPANPSTTFSAAKFASFITQYSTGQVSVEIEWELQKENSKRWNPEIQYTSNYNKSVNVDFTVDTNGVYSEPRPIGTRYLTRNL

SEQ ID NO: 22 - DNA, 2292 bp, Artificial Sequence
  pAAV2-CAP N587 Linker 8 SpyTag HBM  DNA
atggctgccgatggttatcttccagattggctcgaggacactctctctgaaggaataagacagtggtggaagctcaaacctggcccaccaccaccaaagcccgcagagcggcataaggacgacagcaggggtcttgtgcttcctgggtacaagtacctcggacccttcaacggactcgacaagggagagccggtcaacgaggcagacgccgcggccctcgagcacgacaaagcctacgaccggcagctcgacagcggagacaacccgtacctcaagtacaaccacgccgacgcggagtttcaggagcgccttaaagaagatacgtcttttgggggcaacctcggacgagcagtcttccaggcgaaaaagagggttcttgaacctctgggcctggttgaggaacctgttaagacggctccgggaaaaaagaggccggtagagcactctcctgtggagccagactcctcctcgggaaccggaaaggcgggccagcagcctgcaagaaaaagattgaattttggtcagactggagacgcagactcagtacctgacccccagcctctcggacagccaccagcagccccctctggtctgggaactaatacgatggctacaggcagtggcgcaccaatggcagacaataacgagggcgccgacggagtgggtaattcctcgggaaattggcattgcgattccacatggatgggcgacagagtcatcaccaccagcacccgaacctgggccctgcccacctacaacaaccacctctacaaacaaatttccagccaatcaggagcctcgaacgacaatcactactttggctacagcaccccttgggggtattttgacttcaacagattccactgccacttttcaccacgtgactggcaaagactcatcaacaacaactggggattccgacccaagagactcaacttcaagctctttaacattcaagtcaaagaggtcacgcagaatgacggtacgacgacgattgccaataaccttaccagcacggttcaggtgtttactgactcggagtaccagctcccgtacgtcctcggctcggcgcatcaaggatgcctcccgccgttcccagcagacgtcttcatggtgccacagtatggatacctcaccctgaacaacgggagtcaggcagtaggacgctcttcattttactgcctggagtactttccttctcagatgctgcgtaccggaaacaactttaccttcagctacacttttgaggacgttcctttccacagcagctacgctcacagccagagtctggaccgtctcatgaatcctctcatcgaccagtacctgtattacttgagcagaacaaacactccaagtggaaccaccacgcagtcaaggcttcagttttctcaggccggagcgagtgacattcgggaccagtctaggaactggcttcctggaccctgttaccgccagcagcgagtatcaaagacatctgcggataacaacaacagtgaatactcgtggactggagctaccaagtaccacctcaatggcagagactctctggtgaatccgggcccggccatggcaagccacaaggacgatgaagaaaagttttttcctcagagcggggttctcatctttgggaagcaaggctcagagaaaacaaatgtggacattgaaaaggtcatgattacagacgaagaggaaatcaggacaaccaatcccgtggctacggagcagtatggttctgtatctaccaacctccaggcgggcaacggcctgagcggcctgagcggcagcgcccacatcgtgatggtggacgcctacaagccgacgaagggcctgagcggcctgagcggcagccaagcagctaccgcagatgtcaacacacaaggcgttcttccaggcatggtctggcaggacagagatgtgtaccttcaggggcccatctgggcaaagattccacacacggacggacattttcacccctctcccctcatgggtggattcggacttaaacaccctcctccacagattctcatcaagaacaccccggtacctgcgaatccttcgaccaccttcagtgcggcaaagtttgcttccttcatcacacagtactccacgggacaggtcagcgtggagatcgagtgggagctgcagaaggaaaacagcaaacgctggaatcccgaaattcagtacacttccaactacaacaagtctgttaatgtggactttactgtggacactaatggcgtgtattcagagcctcgccccattggcaccagatacctgactcgtaatctgtaa

SEQ ID NO: 23 - protein, 763 aa, Artificial Sequence
  pAAV2-CAP N587 Linker 8 SpyTag HBM  AA
MAADGYLPDWLEDTLSEGIRQWWKLKPGPPPPKPAERHKDDSRGLVLPGYKYLGPFNGLDKGEPVNEADAAALEHDKAYDRQLDSGDNPYLKYNHADAEFQERLKEDTSFGGNLGRAVFQAKKRVLEPLGLVEEPVKTAPGKKRPVEHSPVEPDSSSGTGKAGQQPARKRLNFGQTGDADSVPDPQPLGQPPAAPSGLGTNTMATGSGAPMADNNEGADGVGNSSGNWHCDSTWMGDRVITTSTRTWALPTYNNHLYKQISSQSGASNDNHYFGYSTPWGYFDFNRFHCHFSPRDWQRLINNNWGFRPKRLNFKLFNIQVKEVTQNDGTTTIANNLTSTVQVFTDSEYQLPYVLGSAHQGCLPPFPADVFMVPQYGYLTLNNGSQAVGRSSFYCLEYFPSQMLRTGNNFTFSYTFEDVPFHSSYAHSQSLDRLMNPLIDQYLYYLSRTNTPSGTTTQSRLQFSQAGASDIRDQSRNWLPGPCYRQQRVSKTSADNNNSEYSWTGATKYHLNGRDSLVNPGPAMASHKDDEEKFFPQSGVLIFGKQGSEKTNVDIEKVMITDEEEIRTTNPVATEQYGSVSTNLQAGNGLSGLSGSAHIVMVDAYKPTKGLSGLSGSQAATADVNTQGVLPGMVWQDRDVYLQGPIWAKIPHTDGHFHPSPLMGGFGLKHPPPQILIKNTPVPANPSTTFSAAKFASFITQYSTGQVSVEIEWELQKENSKRWNPEIQYTSNYNKSVNVDFTVDTNGVYSEPRPIGTRYLTRNL

SEQ ID NO: 24 - DNA, 2304 bp, Artificial Sequence
  pAAV2-CAP N587 Linker 10 SpyTag HBM DNA
atggctgccgatggttatcttccagattggctcgaggacactctctctgaaggaataagacagtggtggaagctcaaacctggcccaccaccaccaaagcccgcagagcggcataaggacgacagcaggggtcttgtgcttcctgggtacaagtacctcggacccttcaacggactcgacaagggagagccggtcaacgaggcagacgccgcggccctcgagcacgacaaagcctacgaccggcagctcgacagcggagacaacccgtacctcaagtacaaccacgccgacgcggagtttcaggagcgccttaaagaagatacgtcttttgggggcaacctcggacgagcagtcttccaggcgaaaaagagggttcttgaacctctgggcctggttgaggaacctgttaagacggctccgggaaaaaagaggccggtagagcactctcctgtggagccagactcctcctcgggaaccggaaaggcgggccagcagcctgcaagaaaaagattgaattttggtcagactggagacgcagactcagtacctgacccccagcctctcggacagccaccagcagccccctctggtctgggaactaatacgatggctacaggcagtggcgcaccaatggcagacaataacgagggcgccgacggagtgggtaattcctcgggaaattggcattgcgattccacatggatgggcgacagagtcatcaccaccagcacccgaacctgggccctgcccacctacaacaaccacctctacaaacaaatttccagccaatcaggagcctcgaacgacaatcactactttggctacagcaccccttgggggtattttgacttcaacagattccactgccacttttcaccacgtgactggcaaagactcatcaacaacaactggggattccgacccaagagactcaacttcaagctctttaacattcaagtcaaagaggtcacgcagaatgacggtacgacgacgattgccaataaccttaccagcacggttcaggtgtttactgactcggagtaccagctcccgtacgtcctcggctcggcgcatcaaggatgcctcccgccgttcccagcagacgtcttcatggtgccacagtatggatacctcaccctgaacaacgggagtcaggcagtaggacgctcttcattttactgcctggagtactttccttctcagatgctgcgtaccggaaacaactttaccttcagctacacttttgaggacgttcctttccacagcagctacgctcacagccagagtctggaccgtctcatgaatcctctcatcgaccagtacctgtattacttgagcagaacaaacactccaagtggaaccaccacgcagtcaaggcttcagttttctcaggccggagcgagtgacattcgggaccagtctaggaactggcttcctggaccctgttaccgccagcagcgagtatcaaagacatctgcggataacaacaacagtgaatactcgtggactggagctaccaagtaccacctcaatggcagagactctctggtgaatccgggcccggccatggcaagccacaaggacgatgaagaaaagttttttcctcagagcggggttctcatctttgggaagcaaggctcagagaaaacaaatgtggacattgaaaaggtcatgattacagacgaagaggaaatcaggacaaccaatcccgtggctacggagcagtatggttctgtatctaccaacctccaggcgggcaacggcctgagcggcctgagcggcctgagcggcgcccacatcgtgatggtggacgcctacaagccgacgaagggcctgagcggcctgagcggcctgagcggccaagcagctaccgcagatgtcaacacacaaggcgttcttccaggcatggtctggcaggacagagatgtgtaccttcaggggcccatctgggcaaagattccacacacggacggacattttcacccctctcccctcatgggtggattcggacttaaacaccctcctccacagattctcatcaagaacaccccggtacctgcgaatccttcgaccaccttcagtgcggcaaagtttgcttccttcatcacacagtactccacgggacaggtcagcgtggagatcgagtgggagctgcagaaggaaaacagcaaacgctggaatcccgaaattcagtacacttccaactacaacaagtctgttaatgtggactttactgtggacactaatggcgtgtattcagagcctcgccccattggcaccagatacctgactcgtaatctgtaa

SEQ ID NO: 25 - protein, 767 aa, Artificial Sequence
  pAAV2-CAP N587 Linker 10 SpyTag HBM  AA
MAADGYLPDWLEDTLSEGIRQWWKLKPGPPPPKPAERHKDDSRGLVLPGYKYLGPFNGLDKGEPVNEADAAALEHDKAYDRQLDSGDNPYLKYNHADAEFQERLKEDTSFGGNLGRAVFQAKKRVLEPLGLVEEPVKTAPGKKRPVEHSPVEPDSSSGTGKAGQQPARKRLNFGQTGDADSVPDPQPLGQPPAAPSGLGTNTMATGSGAPMADNNEGADGVGNSSGNWHCDSTWMGDRVITTSTRTWALPTYNNHLYKQISSQSGASNDNHYFGYSTPWGYFDFNRFHCHFSPRDWQRLINNNWGFRPKRLNFKLFNIQVKEVTQNDGTTTIANNLTSTVQVFTDSEYQLPYVLGSAHQGCLPPFPADVFMVPQYGYLTLNNGSQAVGRSSFYCLEYFPSQMLRTGNNFTFSYTFEDVPFHSSYAHSQSLDRLMNPLIDQYLYYLSRTNTPSGTTTQSRLQFSQAGASDIRDQSRNWLPGPCYRQQRVSKTSADNNNSEYSWTGATKYHLNGRDSLVNPGPAMASHKDDEEKFFPQSGVLIFGKQGSEKTNVDIEKVMITDEEEIRTTNPVATEQYGSVSTNLQAGNGLSGLSGLSGAHIVMVDAYKPTKGLSGLSGLSGQAATADVNTQGVLPGMVWQDRDVYLQGPIWAKIPHTDGHFHPSPLMGGFGLKHPPPQILIKNTPVPANPSTTFSAAKFASFITQYSTGQVSVEIEWELQKENSKRWNPEIQYTSNYNKSVNVDFTVDTNGVYSEPRPIGTRYLTRNL

SEQ ID NO: 26 - DNA, 2247 bp, Artificial Sequence
  pAAV2-CAP G453 SpyTag HBM DNA
atggctgccgatggttatcttccagattggctcgaggacactctctctgaaggaataagacagtggtggaagctcaaacctggcccaccaccaccaaagcccgcagagcggcataaggacgacagcaggggtcttgtgcttcctgggtacaagtacctcggacccttcaacggactcgacaagggagagccggtcaacgaggcagacgccgcggccctcgagcacgacaaagcctacgaccggcagctcgacagcggagacaacccgtacctcaagtacaaccacgccgacgcggagtttcaggagcgccttaaagaagatacgtcttttgggggcaacctcggacgagcagtcttccaggcgaaaaagagggttcttgaacctctgggcctggttgaggaacctgttaagacggctccgggaaaaaagaggccggtagagcactctcctgtggagccagactcctcctcgggaaccggaaaggcgggccagcagcctgcaagaaaaagattgaattttggtcagactggagacgcagactcagtacctgacccccagcctctcggacagccaccagcagccccctctggtctgggaactaatacgatggctacaggcagtggcgcaccaatggcagacaataacgagggcgccgacggagtgggtaattcctcgggaaattggcattgcgattccacatggatgggcgacagagtcatcaccaccagcacccgaacctgggccctgcccacctacaacaaccacctctacaaacaaatttccagccaatcaggagcctcgaacgacaatcactactttggctacagcaccccttgggggtattttgacttcaacagattccactgccacttttcaccacgtgactggcaaagactcatcaacaacaactggggattccgacccaagagactcaacttcaagctctttaacattcaagtcaaagaggtcacgcagaatgacggtacgacgacgattgccaataaccttaccagcacggttcaggtgtttactgactcggagtaccagctcccgtacgtcctcggctcggcgcatcaaggatgcctcccgccgttcccagcagacgtcttcatggtgccacagtatggatacctcaccctgaacaacgggagtcaggcagtaggacgctcttcattttactgcctggagtactttccttctcagatgctgcgtaccggaaacaactttaccttcagctacacttttgaggacgttcctttccacagcagctacgctcacagccagagtctggaccgtctcatgaatcctctcatcgaccagtacctgtattacttgagcagaacaaacactccaagtggagcccacatcgtgatggtggacgcctacaagccgacgaagaccaccacgcagtcaaggcttcagttttctcaggccggagcgagtgacattcgggaccagtctaggaactggcttcctggaccctgttacgcccagcaggccgtatcaaagacatctgcggataacaacaacagtgaatactcgtggactggagctaccaagtaccacctcaatggcagagactctctggtgaatccgggcccggccatggcaagccacaaggacgatgaagaagccttttttcctcagagcggggttctcatctttgggaagcaaggctcagagaaaacaaatgtggacattgaaaaggtcatgattacagacgaagaggaaatcaggacaaccaatcccgtggctacggagcagtatggttctgtatctaccaacctccaggccggcaacgcccaagcagctaccgcagatgtcaacacacaaggcgttcttccaggcatggtctggcaggacagagatgtgtaccttcaggggcccatctgggcaaagattccacacacggacggacattttcacccctctcccctcatgggtggattcggacttaaacaccctcctccacagattctcatcaagaacaccccggtacctgcgaatccttcgaccaccttcagtgcggcaaagtttgcttccttcatcacacagtactccacgggacaggtcagcgtggagatcgagtgggagctgcagaaggaaaacagcaaacgctggaatcccgaaattcagtacacttccaactacaacaagtctgttaatgtggactttactgtggacactaatggcgtgtattcagagcctcgccccattggcaccagatacctgactcgtaatctgtaa

SEQ ID NO: 27 - protein, 748 aa, Artificial Sequence
  pAAV2-CAP G453 SpyTag HBM  AA
MAADGYLPDWLEDTLSEGIRQWWKLKPGPPPPKPAERHKDDSRGLVLPGYKYLGPFNGLDKGEPVNEADAAALEHDKAYDRQLDSGDNPYLKYNHADAEFQERLKEDTSFGGNLGRAVFQAKKRVLEPLGLVEEPVKTAPGKKRPVEHSPVEPDSSSGTGKAGQQPARKRLNFGQTGDADSVPDPQPLGQPPAAPSGLGTNTMATGSGAPMADNNEGADGVGNSSGNWHCDSTWMGDRVITTSTRTWALPTYNNHLYKQISSQSGASNDNHYFGYSTPWGYFDFNRFHCHFSPRDWQRLINNNWGFRPKRLNFKLFNIQVKEVTQNDGTTTIANNLTSTVQVFTDSEYQLPYVLGSAHQGCLPPFPADVFMVPQYGYLTLNNGSQAVGRSSFYCLEYFPSQMLRTGNNFTFSYTFEDVPFHSSYAHSQSLDRLMNPLIDQYLYYLSRTNTPSGAHIVMVDAYKPTKTTTQSRLQFSQAGASDIRDQSRNWLPGPCYAQQAVSKTSADNNNSEYSWTGATKYHLNGRDSLVNPGPAMASHKDDEEAFFPQSGVLIFGKQGSEKTNVDIEKVMITDEEEIRTTNPVATEQYGSVSTNLQAGNAQAATADVNTQGVLPGMVWQDRDVYLQGPIWAKIPHTDGHFHPSPLMGGFGLKHPPPQILIKNTPVPANPSTTFSAAKFASFITQYSTGQVSVEIEWELQKENSKRWNPEIQYTSNYNKSVNVDFTVDTNGVYSEPRPIGTRYLTRNL

SEQ ID NO: 28 - DNA, 2307 bp, Artificial Sequence
  pAAV2-CAP G453 Linker10 SpyTag HBM  DNA
atggctgccgatggttatcttccagattggctcgaggacactctctctgaaggaataagacagtggtggaagctcaaacctggcccaccaccaccaaagcccgcagagcggcataaggacgacagcaggggtcttgtgcttcctgggtacaagtacctcggacccttcaacggactcgacaagggagagccggtcaacgaggcagacgccgcggccctcgagcacgacaaagcctacgaccggcagctcgacagcggagacaacccgtacctcaagtacaaccacgccgacgcggagtttcaggagcgccttaaagaagatacgtcttttgggggcaacctcggacgagcagtcttccaggcgaaaaagagggttcttgaacctctgggcctggttgaggaacctgttaagacggctccgggaaaaaagaggccggtagagcactctcctgtggagccagactcctcctcgggaaccggaaaggcgggccagcagcctgcaagaaaaagattgaattttggtcagactggagacgcagactcagtacctgacccccagcctctcggacagccaccagcagccccctctggtctgggaactaatacgatggctacaggcagtggcgcaccaatggcagacaataacgagggcgccgacggagtgggtaattcctcgggaaattggcattgcgattccacatggatgggcgacagagtcatcaccaccagcacccgaacctgggccctgcccacctacaacaaccacctctacaaacaaatttccagccaatcaggagcctcgaacgacaatcactactttggctacagcaccccttgggggtattttgacttcaacagattccactgccacttttcaccacgtgactggcaaagactcatcaacaacaactggggattccgacccaagagactcaacttcaagctctttaacattcaagtcaaagaggtcacgcagaatgacggtacgacgacgattgccaataaccttaccagcacggttcaggtgtttactgactcggagtaccagctcccgtacgtcctcggctcggcgcatcaaggatgcctcccgccgttcccagcagacgtcttcatggtgccacagtatggatacctcaccctgaacaacgggagtcaggcagtaggacgctcttcattttactgcctggagtactttccttctcagatgctgcgtaccggaaacaactttaccttcagctacacttttgaggacgttcctttccacagcagctacgctcacagccagagtctggaccgtctcatgaatcctctcatcgaccagtacctgtattacttgagcagaacaaacactccaagtggaggcctgagcggcctgagcggcctgagcggcgcccacatcgtgatggtggacgcctacaagccgacgaagggcctgagcggcctgagcggcctgagcggcaccaccacgcagtcaaggcttcagttttctcaggccggagcgagtgacattcgggaccagtctaggaactggcttcctggaccctgttacgcccagcaggccgtatcaaagacatctgcggataacaacaacagtgaatactcgtggactggagctaccaagtaccacctcaatggcagagactctctggtgaatccgggcccggccatggcaagccacaaggacgatgaagaagccttttttcctcagagcggggttctcatctttgggaagcaaggctcagagaaaacaaatgtggacattgaaaaggtcatgattacagacgaagaggaaatcaggacaaccaatcccgtggctacggagcagtatggttctgtatctaccaacctccaggccggcaacgcccaagcagctaccgcagatgtcaacacacaaggcgttcttccaggcatggtctggcaggacagagatgtgtaccttcaggggcccatctgggcaaagattccacacacggacggacattttcacccctctcccctcatgggtggattcggacttaaacaccctcctccacagattctcatcaagaacaccccggtacctgcgaatccttcgaccaccttcagtgcggcaaagtttgcttccttcatcacacagtactccacgggacaggtcagcgtggagatcgagtgggagctgcagaaggaaaacagcaaacgctggaatcccgaaattcagtacacttccaactacaacaagtctgttaatgtggactttactgtggacactaatggcgtgtattcagagcctcgccccattggcaccagatacctgactcgtaatctgtaa

SEQ ID NO: 29 - protein, 768 aa, Artificial Sequence
  pAAV2-CAP G453 Linker10 SpyTag HBM  AA
MAADGYLPDWLEDTLSEGIRQWWKLKPGPPPPKPAERHKDDSRGLVLPGYKYLGPFNGLDKGEPVNEADAAALEHDKAYDRQLDSGDNPYLKYNHADAEFQERLKEDTSFGGNLGRAVFQAKKRVLEPLGLVEEPVKTAPGKKRPVEHSPVEPDSSSGTGKAGQQPARKRLNFGQTGDADSVPDPQPLGQPPAAPSGLGTNTMATGSGAPMADNNEGADGVGNSSGNWHCDSTWMGDRVITTSTRTWALPTYNNHLYKQISSQSGASNDNHYFGYSTPWGYFDFNRFHCHFSPRDWQRLINNNWGFRPKRLNFKLFNIQVKEVTQNDGTTTIANNLTSTVQVFTDSEYQLPYVLGSAHQGCLPPFPADVFMVPQYGYLTLNNGSQAVGRSSFYCLEYFPSQMLRTGNNFTFSYTFEDVPFHSSYAHSQSLDRLMNPLIDQYLYYLSRTNTPSGGLSGLSGLSGAHIVMVDAYKPTKGLSGLSGLSGTTTQSRLQFSQAGASDIRDQSRNWLPGPCYAQQAVSKTSADNNNSEYSWTGATKYHLNGRDSLVNPGPAMASHKDDEEAFFPQSGVLIFGKQGSEKTNVDIEKVMITDEEEIRTTNPVATEQYGSVSTNLQAGNAQAATADVNTQGVLPGMVWQDRDVYLQGPIWAKIPHTDGHFHPSPLMGGFGLKHPPPQILIKNTPVPANPSTTFSAAKFASFITQYSTGQVSVEIEWELQKENSKRWNPEIQYTSNYNKSVNVDFTVDTNGVYSEPRPIGTRYLTRNL

SEQ ID NO: 30 - DNA, 2211 bp, Artificial Sequence
  pAAV9-CAP wt DNA
atggctgccgatggttatcttccagattggctcgaggacaaccttagtgaaggaattcgcgagtggtgggctttgaaacctggagcccctcaacccaaggcaaatcaacaacatcaagacaacgctcgaggtcttgtgcttccgggttacaaataccttggacccggcaacggactcgacaagggggagccggtcaacgcagcagacgcggcggccctcgagcacgacaaggcctacgaccagcagctcaaggccggagacaacccgtacctcaagtacaaccacgccgacgccgagttccaggagcggctcaaagaagatacgtcttttgggggcaacctcgggcgagcagtcttccaggccaaaaagaggcttcttgaacctcttggtctggttgaggaagcggctaagacggctcctggaaagaagaggcctgtagagcagtctcctcaggaaccggactcctccgcgggtattggcaaatcgggtgcacagcccgctaaaaagagactcaatttcggtcagactggcgacacagagtcagtcccagaccctcaaccaatcggagaacctcccgcagccccctcaggtgtgggatctcttacaatggcttcaggtggtggcgcaccagtggcagacaataacgaaggtgccgatggagtgggtagttcctcgggaaattggcattgcgattcccaatggctgggggacagagtcatcaccaccagcacccgaacctgggccctgcccacctacaacaatcacctctacaagcaaatctccaacagcacatctggaggatcttcaaatgacaacgcctacttcggctacagcaccccctgggggtattttgacttcaacagattccactgccacttctcaccacgtgactggcagcgactcatcaacaacaactggggattccggcctaagcgactcaacttcaagctcttcaacattcaggtcaaagaggttacggacaacaatggagtcaagaccatcgccaataaccttaccagcacggtccaggtcttcacggactcagactatcagctcccgtacgtgctcgggtcggctcacgagggctgcctcccgccgttcccagcggacgttttcatgattcctcagtacgggtatctgacgcttaatgatggaagccaggccgtgggtcgttcgtccttttactgcctggaatatttcccgtcgcaaatgctaagaacgggtaacaacttccagttcagctacgagtttgagaacgtacctttccatagcagctacgctcacagccaaagcctggaccgactaatgaatccactcatcgaccaatacttgtactatctctcaaagactattaacggttctggacagaatcaacaaacgctaaaattcagtgtggccggacccagcaacatggctgtccagggaagaaactacatacctggacccagctaccgacaacaacgtgtctcaaccactgtgactcaaaacaacaacagcgaatttgcttggcctggagcttcttcttgggctctcaatggacgtaatagcttgatgaatcctggacctgctatggccagccacaaagaaggagaggaccgtttctttcctttgtctggatctttaatttttggcaaacaaggaactggaagagacaacgtggatgcggacaaagtcatgataaccaacgaagaagaaattaaaactactaacccggtagcaacggagtcctatggacaagtggccacaaaccaccagagtgcccaagcacaggcgcagaccggctgggttcaaaaccaaggaatacttccgggtatggtttggcaggacagagatgtgtacctgcaaggacccatttgggccaaaattcctcacacggacggcaactttcacccttctccgctgatgggagggtttggaatgaagcacccgcctcctcagatcctcatcaaaaacacacctgtacctgcggatcctccaacggccttcaacaaggacaagctgaactctttcatcacccagtattctactggccaagtcagcgtggagatcgagtgggagctgcagaaggaaaacagcaagcgctggaacccggagatccagtacacttccaactattacaagtctaataatgttgaatttgctgttaatactgaaggtgtatatagtgaaccccgccccattggcaccagatacctgactcgtaatctgtaa

SEQ ID NO: 31 - protein, 736 aa, adeno-associated virus 9
MAADGYLPDWLEDNLSEGIREWWALKPGAPQPKANQQHQDNARGLVLPGYKYLGPGNGLDKGEPVNAADAAALEHDKAYDQQLKAGDNPYLKYNHADAEFQERLKEDTSFGGNLGRAVFQAKKRLLEPLGLVEEAAKTAPGKKRPVEQSPQEPDSSAGIGKSGAQPAKKRLNFGQTGDTESVPDPQPIGEPPAAPSGVGSLTMASGGGAPVADNNEGADGVGSSSGNWHCDSQWLGDRVITTSTRTWALPTYNNHLYKQISNSTSGGSSNDNAYFGYSTPWGYFDFNRFHCHFSPRDWQRLINNNWGFRPKRLNFKLFNIQVKEVTDNNGVKTIANNLTSTVQVFTDSDYQLPYVLGSAHEGCLPPFPADVFMIPQYGYLTLNDGSQAVGRSSFYCLEYFPSQMLRTGNNFQFSYEFENVPFHSSYAHSQSLDRLMNPLIDQYLYYLSKTINGSGQNQQTLKFSVAGPSNMAVQGRNYIPGPSYRQQRVSTTVTQNNNSEFAWPGASSWALNGRNSLMNPGPAMASHKEGEDRFFPLSGSLIFGKQGTGRDNVDADKVMITNEEEIKTTNPVATESYGQVATNHQSAQAQAQTGWVQNQGILPGMVWQDRDVYLQGPIWAKIPHTDGNFHPSPLMGGFGMKHPPPQILIKNTPVPADPPTAFNKDKLNSFITQYSTGQVSVEIEWELQKENSKRWNPEIQYTSNYYKSNNVEFAVNTEGVYSEPRPIGTRYLTRNL

SEQ ID NO: 32 - DNA, 2211 bp, Artificial Sequence
  pAAV9-CAP W503A DNA
atggctgccgatggttatcttccagattggctcgaggacaaccttagtgaaggaattcgcgagtggtgggctttgaaacctggagcccctcaacccaaggcaaatcaacaacatcaagacaacgctcgaggtcttgtgcttccgggttacaaataccttggacccggcaacggactcgacaagggggagccggtcaacgcagcagacgcggcggccctcgagcacgacaaggcctacgaccagcagctcaaggccggagacaacccgtacctcaagtacaaccacgccgacgccgagttccaggagcggctcaaagaagatacgtcttttgggggcaacctcgggcgagcagtcttccaggccaaaaagaggcttcttgaacctcttggtctggttgaggaagcggctaagacggctcctggaaagaagaggcctgtagagcagtctcctcaggaaccggactcctccgcgggtattggcaaatcgggtgcacagcccgctaaaaagagactcaatttcggtcagactggcgacacagagtcagtcccagaccctcaaccaatcggagaacctcccgcagccccctcaggtgtgggatctcttacaatggcttcaggtggtggcgcaccagtggcagacaataacgaaggtgccgatggagtgggtagttcctcgggaaattggcattgcgattcccaatggctgggggacagagtcatcaccaccagcacccgaacctgggccctgcccacctacaacaatcacctctacaagcaaatctccaacagcacatctggaggatcttcaaatgacaacgcctacttcggctacagcaccccctgggggtattttgacttcaacagattccactgccacttctcaccacgtgactggcagcgactcatcaacaacaactggggattccggcctaagcgactcaacttcaagctcttcaacattcaggtcaaagaggttacggacaacaatggagtcaagaccatcgccaataaccttaccagcacggtccaggtcttcacggactcagactatcagctcccgtacgtgctcgggtcggctcacgagggctgcctcccgccgttcccagcggacgttttcatgattcctcagtacgggtatctgacgcttaatgatggaagccaggccgtgggtcgttcgtccttttactgcctggaatatttcccgtcgcaaatgctaagaacgggtaacaacttccagttcagctacgagtttgagaacgtacctttccatagcagctacgctcacagccaaagcctggaccgactaatgaatccactcatcgaccaatacttgtactatctctcaaagactattaacggttctggacagaatcaacaaacgctaaaattcagtgtggccggacccagcaacatggctgtccagggaagaaactacatacctggacccagctaccgacaacaacgtgtctcaaccactgtgactcaaaacaacaacagcgaatttgctgctcctggagcttcttcttgggctctcaatggacgtaatagcttgatgaatcctggacctgctatggccagccacaaagaaggagaggaccgtttctttcctttgtctggatctttaatttttggcaaacaaggaactggaagagacaacgtggatgcggacaaagtcatgataaccaacgaagaagaaattaaaactactaacccggtagcaacggagtcctatggacaagtggccacaaaccaccagagtgcccaagcacaggcgcagaccggctgggttcaaaaccaaggaatacttccgggtatggtttggcaggacagagatgtgtacctgcaaggacccatttgggccaaaattcctcacacggacggcaactttcacccttctccgctgatgggagggtttggaatgaagcacccgcctcctcagatcctcatcaaaaacacacctgtacctgcggatcctccaacggccttcaacaaggacaagctgaactctttcatcacccagtattctactggccaagtcagcgtggagatcgagtgggagctgcagaaggaaaacagcaagcgctggaacccggagatccagtacacttccaactattacaagtctaataatgttgaatttgctgttaatactgaaggtgtatatagtgaaccccgccccattggcaccagatacctgactcgtaatctgtaa

SEQ ID NO: 33 - protein, 736 aa, Artificial Sequence
  pAAV9-CAP W503A AA
MAADGYLPDWLEDNLSEGIREWWALKPGAPQPKANQQHQDNARGLVLPGYKYLGPGNGLDKGEPVNAADAAALEHDKAYDQQLKAGDNPYLKYNHADAEFQERLKEDTSFGGNLGRAVFQAKKRLLEPLGLVEEAAKTAPGKKRPVEQSPQEPDSSAGIGKSGAQPAKKRLNFGQTGDTESVPDPQPIGEPPAAPSGVGSLTMASGGGAPVADNNEGADGVGSSSGNWHCDSQWLGDRVITTSTRTWALPTYNNHLYKQISNSTSGGSSNDNAYFGYSTPWGYFDFNRFHCHFSPRDWQRLINNNWGFRPKRLNFKLFNIQVKEVTDNNGVKTIANNLTSTVQVFTDSDYQLPYVLGSAHEGCLPPFPADVFMIPQYGYLTLNDGSQAVGRSSFYCLEYFPSQMLRTGNNFQFSYEFENVPFHSSYAHSQSLDRLMNPLIDQYLYYLSKTINGSGQNQQTLKFSVAGPSNMAVQGRNYIPGPSYRQQRVSTTVTQNNNSEFAAPGASSWALNGRNSLMNPGPAMASHKEGEDRFFPLSGSLIFGKQGTGRDNVDADKVMITNEEEIKTTNPVATESYGQVATNHQSAQAQAQTGWVQNQGILPGMVWQDRDVYLQGPIWAKIPHTDGNFHPSPLMGGFGMKHPPPQILIKNTPVPADPPTAFNKDKLNSFITQYSTGQVSVEIEWELQKENSKRWNPEIQYTSNYYKSNNVEFAVNTEGVYSEPRPIGTRYLTRNL

SEQ ID NO: 34 - DNA, 2250 bp, Artificial Sequence
  pAAV9-CAP A589 SpyTag W503A DNA
atggctgccgatggttatcttccagattggctcgaggacaaccttagtgaaggaattcgcgagtggtgggctttgaaacctggagcccctcaacccaaggcaaatcaacaacatcaagacaacgctcgaggtcttgtgcttccgggttacaaataccttggacccggcaacggactcgacaagggggagccggtcaacgcagcagacgcggcggccctcgagcacgacaaggcctacgaccagcagctcaaggccggagacaacccgtacctcaagtacaaccacgccgacgccgagttccaggagcggctcaaagaagatacgtcttttgggggcaacctcgggcgagcagtcttccaggccaaaaagaggcttcttgaacctcttggtctggttgaggaagcggctaagacggctcctggaaagaagaggcctgtagagcagtctcctcaggaaccggactcctccgcgggtattggcaaatcgggtgcacagcccgctaaaaagagactcaatttcggtcagactggcgacacagagtcagtcccagaccctcaaccaatcggagaacctcccgcagccccctcaggtgtgggatctcttacaatggcttcaggtggtggcgcaccagtggcagacaataacgaaggtgccgatggagtgggtagttcctcgggaaattggcattgcgattcccaatggctgggggacagagtcatcaccaccagcacccgaacctgggccctgcccacctacaacaatcacctctacaagcaaatctccaacagcacatctggaggatcttcaaatgacaacgcctacttcggctacagcaccccctgggggtattttgacttcaacagattccactgccacttctcaccacgtgactggcagcgactcatcaacaacaactggggattccggcctaagcgactcaacttcaagctcttcaacattcaggtcaaagaggttacggacaacaatggagtcaagaccatcgccaataaccttaccagcacggtccaggtcttcacggactcagactatcagctcccgtacgtgctcgggtcggctcacgagggctgcctcccgccgttcccagcggacgttttcatgattcctcagtacgggtatctgacgcttaatgatggaagccaggccgtgggtcgttcgtccttttactgcctggaatatttcccgtcgcaaatgctaagaacgggtaacaacttccagttcagctacgagtttgagaacgtacctttccatagcagctacgctcacagccaaagcctggaccgactaatgaatccactcatcgaccaatacttgtactatctctcaaagactattaacggttctggacagaatcaacaaacgctaaaattcagtgtggccggacccagcaacatggctgtccagggaagaaactacatacctggacccagctaccgacaacaacgtgtctcaaccactgtgactcaaaacaacaacagcgaatttgctgctcctggagcttcttcttgggctctcaatggacgtaatagcttgatgaatcctggacctgctatggccagccacaaagaaggagaggaccgtttctttcctttgtctggatctttaatttttggcaaacaaggaactggaagagacaacgtggatgcggacaaagtcatgataaccaacgaagaagaaattaaaactactaacccggtagcaacggagtcctatggacaagtggccacaaaccaccagagtgcccaagcagcccacatcgtgatggtggacgcctacaagccgacgaagcaggcgcagaccggctgggttcaaaaccaaggaatacttccgggtatggtttggcaggacagagatgtgtacctgcaaggacccatttgggccaaaattcctcacacggacggcaactttcacccttctccgctgatgggagggtttggaatgaagcacccgcctcctcagatcctcatcaaaaacacacctgtacctgcggatcctccaacggccttcaacaaggacaagctgaactctttcatcacccagtattctactggccaagtcagcgtggagatcgagtgggagctgcagaaggaaaacagcaagcgctggaacccggagatccagtacacttccaactattacaagtctaataatgttgaatttgctgttaatactgaaggtgtatatagtgaaccccgccccattggcaccagatacctgactcgtaatctgtaa

SEQ ID NO: 35 - protein, 749 aa, Artificial Sequence
  pAAV9-CAP A589 SpyTag W503A AA
MAADGYLPDWLEDNLSEGIREWWALKPGAPQPKANQQHQDNARGLVLPGYKYLGPGNGLDKGEPVNAADAAALEHDKAYDQQLKAGDNPYLKYNHADAEFQERLKEDTSFGGNLGRAVFQAKKRLLEPLGLVEEAAKTAPGKKRPVEQSPQEPDSSAGIGKSGAQPAKKRLNFGQTGDTESVPDPQPIGEPPAAPSGVGSLTMASGGGAPVADNNEGADGVGSSSGNWHCDSQWLGDRVITTSTRTWALPTYNNHLYKQISNSTSGGSSNDNAYFGYSTPWGYFDFNRFHCHFSPRDWQRLINNNWGFRPKRLNFKLFNIQVKEVTDNNGVKTIANNLTSTVQVFTDSDYQLPYVLGSAHEGCLPPFPADVFMIPQYGYLTLNDGSQAVGRSSFYCLEYFPSQMLRTGNNFQFSYEFENVPFHSSYAHSQSLDRLMNPLIDQYLYYLSKTINGSGQNQQTLKFSVAGPSNMAVQGRNYIPGPSYRQQRVSTTVTQNNNSEFAAPGASSWALNGRNSLMNPGPAMASHKEGEDRFFPLSGSLIFGKQGTGRDNVDADKVMITNEEEIKTTNPVATESYGQVATNHQSAQAAHIVMVDAYKPTKQAQTGWVQNQGILPGMVWQDRDVYLQGPIWAKIPHTDGNFHPSPLMGGFGMKHPPPQILIKNTPVPADPPTAFNKDKLNSFITQYSTGQVSVEIEWELQKENSKRWNPEIQYTSNYYKSNNVEFAVNTEGVYSEPRPIGTRYLTRNL

SEQ ID NO: 36 - DNA, 2310 bp, Artificial Sequence
  pAAV9-CAP A589 Linker10 SpyTag W503A DNA
atggctgccgatggttatcttccagattggctcgaggacaaccttagtgaaggaattcgcgagtggtgggctttgaaacctggagcccctcaacccaaggcaaatcaacaacatcaagacaacgctcgaggtcttgtgcttccgggttacaaataccttggacccggcaacggactcgacaagggggagccggtcaacgcagcagacgcggcggccctcgagcacgacaaggcctacgaccagcagctcaaggccggagacaacccgtacctcaagtacaaccacgccgacgccgagttccaggagcggctcaaagaagatacgtcttttgggggcaacctcgggcgagcagtcttccaggccaaaaagaggcttcttgaacctcttggtctggttgaggaagcggctaagacggctcctggaaagaagaggcctgtagagcagtctcctcaggaaccggactcctccgcgggtattggcaaatcgggtgcacagcccgctaaaaagagactcaatttcggtcagactggcgacacagagtcagtcccagaccctcaaccaatcggagaacctcccgcagccccctcaggtgtgggatctcttacaatggcttcaggtggtggcgcaccagtggcagacaataacgaaggtgccgatggagtgggtagttcctcgggaaattggcattgcgattcccaatggctgggggacagagtcatcaccaccagcacccgaacctgggccctgcccacctacaacaatcacctctacaagcaaatctccaacagcacatctggaggatcttcaaatgacaacgcctacttcggctacagcaccccctgggggtattttgacttcaacagattccactgccacttctcaccacgtgactggcagcgactcatcaacaacaactggggattccggcctaagcgactcaacttcaagctcttcaacattcaggtcaaagaggttacggacaacaatggagtcaagaccatcgccaataaccttaccagcacggtccaggtcttcacggactcagactatcagctcccgtacgtgctcgggtcggctcacgagggctgcctcccgccgttcccagcggacgttttcatgattcctcagtacgggtatctgacgcttaatgatggaagccaggccgtgggtcgttcgtccttttactgcctggaatatttcccgtcgcaaatgctaagaacgggtaacaacttccagttcagctacgagtttgagaacgtacctttccatagcagctacgctcacagccaaagcctggaccgactaatgaatccactcatcgaccaatacttgtactatctctcaaagactattaacggttctggacagaatcaacaaacgctaaaattcagtgtggccggacccagcaacatggctgtccagggaagaaactacatacctggacccagctaccgacaacaacgtgtctcaaccactgtgactcaaaacaacaacagcgaatttgctgctcctggagcttcttcttgggctctcaatggacgtaatagcttgatgaatcctggacctgctatggccagccacaaagaaggagaggaccgtttctttcctttgtctggatctttaatttttggcaaacaaggaactggaagagacaacgtggatgcggacaaagtcatgataaccaacgaagaagaaattaaaactactaacccggtagcaacggagtcctatggacaagtggccacaaaccaccagagtgcccaagcaggcctgagcagcggcagcggcctgagcggcgcccacatcgtgatggtggacgcctacaagccgacgaagggcctgagcggcggcagcggcctgagcggccaggcgcagaccggctgggttcaaaaccaaggaatacttccgggtatggtttggcaggacagagatgtgtacctgcaaggacccatttgggccaaaattcctcacacggacggcaactttcacccttctccgctgatgggagggtttggaatgaagcacccgcctcctcagatcctcatcaaaaacacacctgtacctgcggatcctccaacggccttcaacaaggacaagctgaactctttcatcacccagtattctactggccaagtcagcgtggagatcgagtgggagctgcagaaggaaaacagcaagcgctggaacccggagatccagtacacttccaactattacaagtctaataatgttgaatttgctgttaatactgaaggtgtatatagtgaaccccgccccattggcaccagatacctgactcgtaatctgtaa

SEQ ID NO: 37 - protein, 769 aa, Artificial Sequence
  pAAV9-CAP A589 Linker10 SpyTag W503A AA
MAADGYLPDWLEDNLSEGIREWWALKPGAPQPKANQQHQDNARGLVLPGYKYLGPGNGLDKGEPVNAADAAALEHDKAYDQQLKAGDNPYLKYNHADAEFQERLKEDTSFGGNLGRAVFQAKKRLLEPLGLVEEAAKTAPGKKRPVEQSPQEPDSSAGIGKSGAQPAKKRLNFGQTGDTESVPDPQPIGEPPAAPSGVGSLTMASGGGAPVADNNEGADGVGSSSGNWHCDSQWLGDRVITTSTRTWALPTYNNHLYKQISNSTSGGSSNDNAYFGYSTPWGYFDFNRFHCHFSPRDWQRLINNNWGFRPKRLNFKLFNIQVKEVTDNNGVKTIANNLTSTVQVFTDSDYQLPYVLGSAHEGCLPPFPADVFMIPQYGYLTLNDGSQAVGRSSFYCLEYFPSQMLRTGNNFQFSYEFENVPFHSSYAHSQSLDRLMNPLIDQYLYYLSKTINGSGQNQQTLKFSVAGPSNMAVQGRNYIPGPSYRQQRVSTTVTQNNNSEFAAPGASSWALNGRNSLMNPGPAMASHKEGEDRFFPLSGSLIFGKQGTGRDNVDADKVMITNEEEIKTTNPVATESYGQVATNHQSAQAGLSSGSGLSGAHIVMVDAYKPTKGLSGGSGLSGQAQTGWVQNQGILPGMVWQDRDVYLQGPIWAKIPHTDGNFHPSPLMGGFGMKHPPPQILIKNTPVPADPPTAFNKDKLNSFITQYSTGQVSVEIEWELQKENSKRWNPEIQYTSNYYKSNNVEFAVNTEGVYSEPRPIGTRYLTRNL

SEQ ID NO: 38 - DNA, 2310 bp, Artificial Sequence
  pAAV9-CAP G453 Linker10 SpyTag W503A  DNA
atggctgccgatggttatcttccagattggctcgaggacaaccttagtgaaggaattcgcgagtggtgggctttgaaacctggagcccctcaacccaaggcaaatcaacaacatcaagacaacgctcgaggtcttgtgcttccgggttacaaataccttggacccggcaacggactcgacaagggggagccggtcaacgcagcagacgcggcggccctcgagcacgacaaggcctacgaccagcagctcaaggccggagacaacccgtacctcaagtacaaccacgccgacgccgagttccaggagcggctcaaagaagatacgtcttttgggggcaacctcgggcgagcagtcttccaggccaaaaagaggcttcttgaacctcttggtctggttgaggaagcggctaagacggctcctggaaagaagaggcctgtagagcagtctcctcaggaaccggactcctccgcgggtattggcaaatcgggtgcacagcccgctaaaaagagactcaatttcggtcagactggcgacacagagtcagtcccagaccctcaaccaatcggagaacctcccgcagccccctcaggtgtgggatctcttacaatggcttcaggtggtggcgcaccagtggcagacaataacgaaggtgccgatggagtgggtagttcctcgggaaattggcattgcgattcccaatggctgggggacagagtcatcaccaccagcacccgaacctgggccctgcccacctacaacaatcacctctacaagcaaatctccaacagcacatctggaggatcttcaaatgacaacgcctacttcggctacagcaccccctgggggtattttgacttcaacagattccactgccacttctcaccacgtgactggcagcgactcatcaacaacaactggggattccggcctaagcgactcaacttcaagctcttcaacattcaggtcaaagaggttacggacaacaatggagtcaagaccatcgccaataaccttaccagcacggtccaggtcttcacggactcagactatcagctcccgtacgtgctcgggtcggctcacgagggctgcctcccgccgttcccagcggacgttttcatgattcctcagtacgggtatctgacgcttaatgatggaagccaggccgtgggtcgttcgtccttttactgcctggaatatttcccgtcgcaaatgctaagaacgggtaacaacttccagttcagctacgagtttgagaacgtacctttccatagcagctacgctcacagccaaagcctggaccgactaatgaatccactcatcgaccaatacttgtactatctctcaaagactattaacggtggcctgagcagcggcagcggcctgagcggcgcccacatcgtgatggtggacgcctacaagccgacgaagggcctgagcggcggcagcggcctgagcggctctggacagaatcaacaaacgctaaaattcagtgtggccggacccagcaacatggctgtccagggaagaaactacatacctggacccagctaccgacaacaacgtgtctcaaccactgtgactcaaaacaacaacagcgaatttgctgctcctggagcttcttcttgggctctcaatggacgtaatagcttgatgaatcctggacctgctatggccagccacaaagaaggagaggaccgtttctttcctttgtctggatctttaatttttggcaaacaaggaactggaagagacaacgtggatgcggacaaagtcatgataaccaacgaagaagaaattaaaactactaacccggtagcaacggagtcctatggacaagtggccacaaaccaccagagtgcccaagcacaggcgcagaccggctgggttcaaaaccaaggaatacttccgggtatggtttggcaggacagagatgtgtacctgcaaggacccatttgggccaaaattcctcacacggacggcaactttcacccttctccgctgatgggagggtttggaatgaagcacccgcctcctcagatcctcatcaaaaacacacctgtacctgcggatcctccaacggccttcaacaaggacaagctgaactctttcatcacccagtattctactggccaagtcagcgtggagatcgagtgggagctgcagaaggaaaacagcaagcgctggaacccggagatccagtacacttccaactattacaagtctaataatgttgaatttgctgttaatactgaaggtgtatatagtgaaccccgccccattggcaccagatacctgactcgtaatctgtaa

SEQ ID NO: 39 - protein, 769 aa, Artificial Sequence
  pAAV9-RC G453 Linker10 SpyTag W503A  AA
MAADGYLPDWLEDNLSEGIREWWALKPGAPQPKANQQHQDNARGLVLPGYKYLGPGNGLDKGEPVNAADAAALEHDKAYDQQLKAGDNPYLKYNHADAEFQERLKEDTSFGGNLGRAVFQAKKRLLEPLGLVEEAAKTAPGKKRPVEQSPQEPDSSAGIGKSGAQPAKKRLNFGQTGDTESVPDPQPIGEPPAAPSGVGSLTMASGGGAPVADNNEGADGVGSSSGNWHCDSQWLGDRVITTSTRTWALPTYNNHLYKQISNSTSGGSSNDNAYFGYSTPWGYFDFNRFHCHFSPRDWQRLINNNWGFRPKRLNFKLFNIQVKEVTDNNGVKTIANNLTSTVQVFTDSDYQLPYVLGSAHEGCLPPFPADVFMIPQYGYLTLNDGSQAVGRSSFYCLEYFPSQMLRTGNNFQFSYEFENVPFHSSYAHSQSLDRLMNPLIDQYLYYLSKTINGGLSSGSGLSGAHIVMVDAYKPTKGLSGGSGLSGSGQNQQTLKFSVAGPSNMAVQGRNYIPGPSYRQQRVSTTVTQNNNSEFAAPGASSWALNGRNSLMNPGPAMASHKEGEDRFFPLSGSLIFGKQGTGRDNVDADKVMITNEEEIKTTNPVATESYGQVATNHQSAQAQAQTGWVQNQGILPGMVWQDRDVYLQGPIWAKIPHTDGNFHPSPLMGGFGMKHPPPQILIKNTPVPADPPTAFNKDKLNSFITQYSTGQVSVEIEWELQKENSKRWNPEIQYTSNYYKSNNVEFAVNTEGVYSEPRPIGTRYLTRNL

SEQ ID NO: 40 - protein, 4 aa, Artificial Sequence
  4 linker
GLSG

SEQ ID NO: 41 - protein, 6 aa, Artificial Sequence
  6 linker
GLSGSG

SEQ ID NO: 42 - protein, 8 aa, Artificial Sequence
  8 linker
GLSGLSGS

SEQ ID NO: 43 - protein, 10 aa, Artificial Sequence
  10 linker
GLSGLSGLSG

SEQ ID NO: 44 - protein, 10 aa, Artificial Sequence
  10 linker SEQ ID NO:44
GLSGGSGLSG

SEQ ID NO: 45 - DNA, 1341 bp, Artificial Sequence
  Human IgG4 heavy chain - linker - SpyCatcher
gcctccaccaagggcccatcggtcttccccctggcgccctgctccaggagcacctccgagagcacagccgccctgggctgcctggtcaaggactacttccccgaaccggtgacggtgtcgtggaactcaggcgccctgaccagcggcgtgcacaccttcccggctgtcctacagtcctcaggactctactccctcagcagcgtggtgaccgtgccctccagcagcttgggcacgaagacctacacctgcaacgtagatcacaagcccagcaacaccaaggtggacaagagagttgagtccaaatatggtcccccatgcccaccctgcccagcacctgagttcctggggggaccatcagtcttcctgttccccccaaaacccaaggacactctcatgatctcccggacccctgaggtcacgtgcgtggtggtggacgtgagccaggaagaccccgaggtccagttcaactggtacgtggatggcgtggaggtgcataatgccaagacaaagccgcgggaggagcagttcaacagcacgtaccgtgtggtcagcgtcctcaccgtcctgcaccaggactggctgaacggcaaggagtacaagtgcaaggtctccaacaaaggcctcccgtcctccatcgagaaaaccatctccaaagccaaagggcagccccgagagccacaggtgtacaccctgcccccatcccaggaggagatgaccaagaaccaggtcagcctgacctgcctggtcaaaggcttctaccccagcgacatcgccgtggagtgggagagcaatgggcagccggagaacaactacaagaccacgcctcccgtgctggactccgacggctccttcttcctctacagcaggctcaccgtggacaagagcaggtggcaggaggggaatgtcttctcatgctccgtgatgcatgaggctctgcacaaccactacacacagaagtccctctccctgtctctgggtaaaggaagcggcgaaagcggcgtggataccctgtccggactgagcagtgagcaaggccagtccggagatatgacaattgaagaagatagcgccacccatattaaattctccaaaagagatgaggacggcaaagagctggctggagcaacaatggagctgagagattcctctggaaagactattagtacatggatctctgatggccaagtgaaagatttctatctgtatccaggaaagtacacatttgtcgaaaccgctgcaccagacggatatgaggtggctacagctattacctttacagtgaatgagcaaggacaggtgactgttaatggcaaagctactaaaggagacgctcatatttaa

SEQ ID NO: 46 - protein, 446 aa, Artificial Sequence
  SEQ ID NO:46
ASTKGPSVFPLAPCSRSTSESTAALGCLVKDYFPEPVTVSWNSGALTSGVHTFPAVLQSSGLYSLSSVVTVPSSSLGTKTYTCNVDHKPSNTKVDKRVESKYGPPCPPCPAPEFLGGPSVFLFPPKPKDTLMISRTPEVTCVVVDVSQEDPEVQFNWYVDGVEVHNAKTKPREEQFNSTYRVVSVLTVLHQDWLNGKEYKCKVSNKGLPSSIEKTISKAKGQPREPQVYTLPPSQEEMTKNQVSLTCLVKGFYPSDIAVEWESNGQPENNYKTTPPVLDSDGSFFLYSRLTVDKSRWQEGNVFSCSVMHEALHNHYTQKSLSLSLGKGSGESGVDTLSGLSSEQGQSGDMTIEEDSATHIKFSKRDEDGKELAGATMELRDSSGKTISTWISDGQVKDFYLYPGKYTFVETAAPDGYEVATAITFTVNEQGQVTVNGKATKGDAHI

SEQ ID NO: 47 - DNA, 18 bp, Artificial Sequence
  IgG-SpyCatcher Linker DNA
ggaagcggcgaaagcggc

SEQ ID NO: 48 - protein, 6 aa, Artificial Sequence
  IgG-SpyCatcher Linker AA
GSGESG

SEQ ID NO: 49 - DNA, 1020 bp, Artificial Sequence
  IgG
gcctccaccaagggcccatcggtcttccccctggcgccctgctccaggagcacctccgagagcacagccgccctgggctgcctggtcaaggactacttccccgaaccggtgacggtgtcgtggaactcaggcgccctgaccagcggcgtgcacaccttcccggctgtcctacagtcctcaggactctactccctcagcagcgtggtgaccgtgccctccagcagcttgggcacgaagacctacacctgcaacgtagatcacaagcccagcaacaccaaggtggacaagagagttgagtccaaatatggtcccccatgcccaccctgcccagcacctgagttcctggggggaccatcagtcttcctgttccccccaaaacccaaggacactctcatgatctcccggacccctgaggtcacgtgcgtggtggtggacgtgagccaggaagaccccgaggtccagttcaactggtacgtggatggcgtggaggtgcataatgccaagacaaagccgcgggaggagcagttcaacagcacgtaccgtgtggtcagcgtcctcaccgtcctgcaccaggactggctgaacggcaaggagtacaagtgcaaggtctccaacaaaggcctcccgtcctccatcgagaaaaccatctccaaagccaaagggcagccccgagagccacaggtgtacaccctgcccccatcccaggaggagatgaccaagaaccaggtcagcctgacctgcctggtcaaaggcttctaccccagcgacatcgccgtggagtgggagagcaatgggcagccggagaacaactacaagaccacgcctcccgtgctggactccgacggctccttcttcctctacagcaggctcaccgtggacaagagcaggtggcaggaggggaatgtcttctcatgctccgtgatgcatgaggctctgcacaaccactacacacagaagtccctctccctgtctctgggtaaaggaagcggcgaaagcggcgtggataccctgtccggactg

SEQ ID NO: 50 - protein, 327 aa, Artificial Sequence
  IgG AA
ASTKGPSVFPLAPCSRSTSESTAALGCLVKDYFPEPVTVSWNSGALTSGVHTFPAVLQSSGLYSLSSVVTVPSSSLGTKTYTCNVDHKPSNTKVDKRVESKYGPPCPPCPAPEFLGGPSVFLFPPKPKDTLMISRTPEVTCVVVDVSQEDPEVQFNWYVDGVEVHNAKTKPREEQFNSTYRVVSVLTVLHQDWLNGKEYKCKVSNKGLPSSIEKTISKAKGQPREPQVYTLPPSQEEMTKNQVSLTCLVKGFYPSDIAVEWESNGQPENNYKTTPPVLDSDGSFFLYSRLTVDKSRWQEGNVFSCSVMHEALHNHYTQKSLSLSLGK

SEQ ID NO: 51 - protein, 736 aa, adeno-associated virus 6
MAADGYLPDWLEDNLSEGIREWWDLKPGAPKPKANQQKQDDGRGLVLPGYKYLGPFNGLDKGEPVNAADAAALEHDKAYDQQLKAGDNPYLRYNHADAEFQERLQEDTSFGGNLGRAVFQAKKRVLEPFGLVEEGAKTAPGKKRPVEQSPQEPDSSSGIGKTGQQPAKKRLNFGQTGDSESVPDPQPLGEPPATPAAVGPTTMASGGGAPMADNNEGADGVGNASGNWHCDSTWLGDRVITTSTRTWALPTYNNHLYKQISSASTGASNDNHYFGYSTPWGYFDFNRFHCHFSPRDWQRLINNNWGFRPKRLNFKLFNIQVKEVTTNDGVTTIANNLTSTVQVFSDSEYQLPYVLGSAHQGCLPPFPADVFMIPQYGYLTLNNGSQAVGRSSFYCLEYFPSQMLRTGNNFTFSYTFEDVPFHSSYAHSQSLDRLMNPLIDQYLYYLNRTQNQSGSAQNKDLLFSRGSPAGMSVQPKNWLPGPCYRQQRVSKTKTDNNNSNFTWTGASKYNLNGRESIINPGTAMASHKDDKDKFFPMSGVMIFGKESAGASNTALDNVMITDEEEIKATNPVATERFGTVAVNLQSSSTDPATGDVHVMGALPGMVWQDRDVYLQGPIWAKIPHTDGHFHPSPLMGGFGLKHPPPQILIKNTPVPANPPAEFSATKFASFITQYSTGQVSVEIEWELQKENSKRWNPEVQYTSNYAKSANVDFTVDNNGLYTEPRPIGTRYLTRPL

SEQ ID NO: 52 - DNA, 2238 bp, Artificial Sequence
  encodes pAAV2N587Myc
atggctgccgatggttatcttccagattggctcgaggacactctctctgaaggaataagacagtggtggaagctcaaacctggcccaccaccaccaaagcccgcagagcggcataaggacgacagcaggggtcttgtgcttcctgggtacaagtacctcggacccttcaacggactcgacaagggagagccggtcaacgaggcagacgccgcggccctcgagcacgacaaagcctacgaccggcagctcgacagcggagacaacccgtacctcaagtacaaccacgccgacgcggagtttcaggagcgccttaaagaagatacgtcttttgggggcaacctcggacgagcagtcttccaggcgaaaaagagggttcttgaacctctgggcctggttgaggaacctgttaagacggctccgggaaaaaagaggccggtagagcactctcctgtggagccagactcctcctcgggaaccggaaaggcgggccagcagcctgcaagaaaaagattgaattttggtcagactggagacgcagactcagtacctgacccccagcctctcggacagccaccagcagccccctctggtctgggaactaatacgatggctacaggcagtggcgcaccaatggcagacaataacgagggcgccgacggagtgggtaattcctcgggaaattggcattgcgattccacatggatgggcgacagagtcatcaccaccagcacccgaacctgggccctgcccacctacaacaaccacctctacaaacaaatttccagccaatcaggagcctcgaacgacaatcactactttggctacagcaccccttgggggtattttgacttcaacagattccactgccacttttcaccacgtgactggcaaagactcatcaacaacaactggggattccgacccaagagactcaacttcaagctctttaacattcaagtcaaagaggtcacgcagaatgacggtacgacgacgattgccaataaccttaccagcacggttcaggtgtttactgactcggagtaccagctcccgtacgtcctcggctcggcgcatcaaggatgcctcccgccgttcccagcagacgtcttcatggtgccacagtatggatacctcaccctgaacaacgggagtcaggcagtaggacgctcttcattttactgcctggagtactttccttctcagatgctgcgtaccggaaacaactttaccttcagctacacttttgaggacgttcctttccacagcagctacgctcacagccagagtctggaccgtctcatgaatcctctcatcgaccagtacctgtattacttgagcagaacaaacactccaagtggaaccaccacgcagtcaaggcttcagttttctcaggccggagcgagtgacattcgggaccagtctaggaactggcttcctggaccctgttaccgccagcagcgagtatcaaagacatctgcggataacaacaacagtgaatactcgtggactggagctaccaagtaccacctcaatggcagagactctctggtgaatccgggcccggccatggcaagccacaaggacgatgaagaaaagttttttcctcagagcggggttctcatctttgggaagcaaggctcagagaaaacaaatgtggacattgaaaaggtcatgattacagacgaagaggaaatcaggacaaccaatcccgtggctacggagcagtatggttctgtatctaccaacctccagagaggcaacgaacaaaaactcatctcagaagaggatctgagacaagcagctaccgcagatgtcaacacacaaggcgttcttccaggcatggtctggcaggacagagatgtgtaccttcaggggcccatctgggcaaagattccacacacggacggacattttcacccctctcccctcatgggtggattcggacttaaacaccctcctccacagattctcatcaagaacaccccggtacctgcgaatccttcgaccaccttcagtgcggcaaagtttgcttccttcatcacacagtactccacgggacaggtcagcgtggagatcgagtgggagctgcagaaggaaaacagcaaacgctggaatcccgaaattcagtacacttccaactacaacaagtctgttaatgtggactttactgtggacactaatggcgtgtattcagagcctcgccccattggcaccagatacctgactcgtaatctgtaa

SEQ ID NO: 53 - protein, 745 aa, Artificial Sequence
  Amino acid sequence of pAAV2N587 Myc
MAADGYLPDWLEDTLSEGIRQWWKLKPGPPPPKPAERHKDDSRGLVLPGYKYLGPFNGLDKGEPVNEADAAALEHDKAYDRQLDSGDNPYLKYNHADAEFQERLKEDTSFGGNLGRAVFQAKKRVLEPLGLVEEPVKTAPGKKRPVEHSPVEPDSSSGTGKAGQQPARKRLNFGQTGDADSVPDPQPLGQPPAAPSGLGTNTMATGSGAPMADNNEGADGVGNSSGNWHCDSTWMGDRVITTSTRTWALPTYNNHLYKQISSQSGASNDNHYFGYSTPWGYFDFNRFHCHFSPRDWQRLINNNWGFRPKRLNFKLFNIQVKEVTQNDGTTTIANNLTSTVQVFTDSEYQLPYVLGSAHQGCLPPFPADVFMVPQYGYLTLNNGSQAVGRSSFYCLEYFPSQMLRTGNNFTFSYTFEDVPFHSSYAHSQSLDRLMNPLIDQYLYYLSRTNTPSGTTTQSRLQFSQAGASDIRDQSRNWLPGPCYRQQRVSKTSADNNNSEYSWTGATKYHLNGRDSLVNPGPAMASHKDDEEKFFPQSGVLIFGKQGSEKTNVDIEKVMITDEEEIRTTNPVATEQYGSVSTNLQRGNEQKLISEEDLRQAATADVNTQGVLPGMVWQDRDVYLQGPIWAKIPHTDGHFHPSPLMGGFGLKHPPPQILIKNTPVPANPSTTFSAAKFASFITQYSTGQVSVEIEWELQKENSKRWNPEIQYTSNYNKSVNVDFTVDTNGVYSEPRPIGTRYLTRNL

SEQ ID NO: 54 - protein, 14 aa, Artificial Sequence
  SpyTag002
VPTIVMVDAYKRYK

SEQ ID NO: 55 - protein, 113 aa, Artificial Sequence
  SpyCatcher002
VTTLSGLSGEQGPSGDMTTEEDSATHIKFSKRDEDGRELAGATMELRDSSGKTISTWISDGHVKDFYLYPGKYTFVETAAPDGYEVATAITFTVNEQGQVTVNGEATKGDAHT